European Patent Specification EP 4 168 582 B1, published November 19, 2025. Title: SELECTION METHOD. Applicant: OXFORD NANOPORE TECHNOLOGIES LIMITED. The sequence listing filed with the application follows.

SEQUENCE LISTING (47 sequences)

SEQ ID NO: 1 - protein, 485 aa, Escherichia coli
MMNDGKQQSTFLFHDYETFGTHPALDRPAQFAAIRTDSEFNVIGEPEVFYCKPADDYLPQPGAVLITGITPQEARAKGENEAAFAARIHSLFTVPKTCILGYNNVRFDDEVTRNIFYRNFYDPYAWSWQHDNSRWDLLDVMRACYALRPEGINWPENDDGLPSFRLEHLTKANGIEHSNAHDAMADVYATIAMAKLVKTRQPRLFDYLFTHRNKHKLMALIDVPQMKPLVHVSGMFGAWRGNTSWVAPLAWHPENRNAVIMVDLAGDISPLLELDSDTLRERLYTAKTDLGDNAAVPVKLVHINKCPVLAQANTLRPEDADRLGINRQHCLDNLKILRENPQVREKVVAIFAEAEPFTPSDNVDAQLYNGFFSDADRAAMKIVLETEPRNLPALDITFVDKRIEKLLFNYRARNFPGTLDYAEQQRWLEHRRQVFTPEFLQGYADELQMLVQQYADDKEKVALLKALWQYAEEIVSGSGHHHHHH

SEQ ID NO: 2 - protein, 268 aa, Escherichia coli
MKFVSFNINGLRARPHQLEAIVEKHQPDVIGLQETKVHDDMFPLEEVAKLGYNVFYHGQKGHYGVALLTKETPIAVRRGFPGDDEEAQRRIIMAEIPSLLGNVTVINGYFPQGESRDHPIKFPAKAQFYQNLQNYLETELKRDNPVLIMGDMNISPTDLDIGIGEENRKRWLRTGKCSFLPEEREWMDRLMSWGLVDTFRHANPQTADRFSWFDYRSKGFDDNRGLRIDLLLASQPLAECCVETGIDYEIRSMEKPSDHAPVWATFRR

SEQ ID NO: 3 - protein, 425 aa, Thermus thermophilus
MFRRKEDLDPPLALLPLKGLREAAALLEEALRQGKRIRVHGDYDADGLTGTAILVRGLAALGADVHPFIPHRLEEGYGVLMERVPEHLEASDLFLTVDCGITNHAELRELLENGVEVIVTDHHTPGKTPPPGLVVHPALTPDLKEKPTGAGVAFLLLWALHERLGLPPPLEYADLAAVGTIADVAPLWGWNRALVKEGLARIPASSWVGLRLLAEAVGYTGKAVEVAFRIAPRINAASRLGEAEKALRLLLTDDAAEAQALVGELHRLNARRQTLEEAMLRKLLPQADPEAKAIVLLDPEGHPGVMGIVASRILEATLRPVFLVAQGKGTVRSLAPISAVEALRSAEDLLLRYGGHKEAAGFAMDEALFPAFKARVEAYAARFPDPVREVALLDLLPEPGLLPQVFRELALLEPYGEGNPEPLFL

SEQ ID NO: 4 - protein, 226 aa, Bacteriophage lambda
MTPDIILQRTGIDVRAVEQGDDAWHKLRLGVITASEVHNVIAKPRSGKKWPDMKMSYFHTLLAEVCTGVAPEVNAKALAWGKQYENDARTLFEFTSGVNVTESPIIYRDESMRTACSPDGLCSDGNGLELKCPFTSRDFMKFRLGGFEAIKSAYMAQVQYSMWVTRKNAWYFANYDPRMKREGLHYVVIERDEKYMASFDEIVPEFIEKMDEALAEIGFVFGEQWR

SEQ ID NO: 5 - protein, 608 aa, Bacillus subtilis
MKHMPRKMYSCAFETTTKVEDCRVWAYGYMNIEDHSEYKIGNSLDEFMAWVLKVQADLYFHNLKFDGAFIINWLERNGFKWSADGLPNTYNTIISRMGQWYMIDICLGYKGKRKIHTVIYDSLKKLPFPVKKIAKDFKLTVLKGDIDYHKERPVGYKITPEEYAYIKNDIQIIAEALLIQFKQGLDRMTAGSDSLKGFKDIITTKKFKKVFPTLSLGLDKEVRYAYRGGFTWLNDRFKEKEIGEGMVFDVNSLYPAQMYSRLLPYGEPIVFEGKYVWDEDYPLHIQHIRCEFELKEGYIPTIQIKRSRFYKGNEYLKSSGGEIADLWLSNVDLELMKEHYDLYNVEYISGLKFKATTGLFKDFIDKWTYIKTTSEGAIKQLAKLMLNSLYGKFASNPDVTGKVPYLKENGALGFRLGEEETKDPVYTPMGVFITAWARYTTITAAQACYDRIIYCDTDSIHLTGTEIPDVIKDIVDPKKLGYWAHESTFKRAKYLRQKTYIQDIYMKEVDGKLVEGSPDDYTDIKFSVKCAGMTDKIKKEVTFENFKVGFSRKMKPKPVQVPGGVVLVDDTFTIKSGGSAWSHPQFEKGGGSGGGSGGSAWSHPQFEK

SEQ ID NO: 6 - protein, 970 aa, Citromicrobium bathyomarinum
MLSVANVRSPSAAASYFASDNYYASADADRSGQWIGDGAKRLGLEGKVEARAFDALLRGELPDGSSVGNPGQAHRPGTDLTFSVPKSWSLLALVGKDERIIAAYREAVVEALHWAEKNAAETRVVEKGMVVTQATGNLAIGLFQHDTNRNQEPNLHFHAVIANVTQGKDGKWRTLKNDRLWQLNTTLNSIAMARFRVAVEKLGYEPGPVLKHGNFEARGISREQVMAFSTRRKEVLEARRGPGLDAGRIAALDTRASKEGIEDRATLSKQWSEAAQSIGLDLKPLVDRARTKALGQGMEATRIGSLVERGRAWLSRFAAHVRGDPADPLVPPSVLKQDRQTIAAAQAVASAVRHLSQREAAFERTALYKAALDFGLPTTIADVEKRTRALVRSGDLIAGKGEHKGWLASRDAVVTEQRILSEVAAGKGDSSPAITPQKAAASVQAAALTGQGFRLNEGQLAAARLILISKDRTIAVQGIAGAGKSSVLKPVAEVLRDEGHPVIGLAIQNTLVQMLERDTGIGSQTLARFLGGWNKLLDDPGNVALRAEAQASLKDHVLVLDEASMVSNEDKEKLVRLANLAGVHRLVLIGDRKQLGAVDAGKPFALLQRAGIARAEMATNLRARDPVVREAQAAAQAGDVRKALRHLKSHTVEARGDGAQVAAETWLALDKETRARTSIYASGRAIRSAVNAAVQQGLLASREIGPAKMKLEVLDRVNTTREELRHLPAYRAGRVLEVSRKQQALGLFIGEYRVIGQDRKGKLVEVEDKRGKRFRFDPARIRAGKGDDNLTLLEPRKLEIHEGDRIRWTRNDHRRGLFNADQARVVEIANGKVTFETSKGDLVELKKDDPMLKRIDLAYALNVHMAQGLTSDRGIAVMDSRERNLSNQKTFLVTVTRLRDHLTLVVDSADKLGAAVARNKGEKASAIEVTGSVKPTATKGSGVDQPKSVEANKAEKELTRSKSKTLDFGI

SEQ ID NO: 7 - protein, 760 aa, Methanococcoides burtonii
MMIRELDIPRDIIGFYEDSGIKELYPPQAEAIEMGLLEKKNLLAAIPTASGKTLLAELAMIKAIREGGKALYIVPLRALASEKFERFKELAPFGIKVGISTGDLDSRADWLGVNDIIVATSEKTDSLLRNGTSWMDEITTVVVDEIHLLDSKNRGPTLEVTITKLMRLNPDVQVVALSATVGNAREMADWLGAALVLSEWRPTDLHEGVLFGDAINFPGSQKKIDRLEKDDAVNLVLDTIKAEGQCLVFESSRRNCAGFAKTASSKVAKILDNDIMIKLAGIAEEVESTGETDTAIVLANCIRKGVAFHHAGLNSNHRKLVENGFRQNLIKVISSTPTLAAGLNLPARRVIIRSYRRFDSNFGMQPIPVLEYKQMAGRAGRPHLDPYGESVLLAKTYDEFAQLMENYVEADAEDIWSKLGTENALRTHVLSTIVNGFASTRQELFDFFGATFFAYQQDKWMLEEVINDCLEFLIDKAMVSETEDIEDASKLFLRGTRLGSLVSMLYIDPLSGSKIVDGFKDIGKSTGGNMGSLEDDKGDDITVTDMTLLHLVCSTPDMRQLYLRNTDYTIVNEYIVAHSDEFHEIPDKLKETDYEWFMGEVKTAMLLEEWVTEVSAEDITRHFNVGEGDIHALADTSEWLMHAAAKLAELLGVEYSSHAYSLEKRIRYGSGLDLMELVGIRGVGRVRARKLYNAGFVSVAKLKGADISVLSKLVGPKVAYNILSGIGVRVNDKHFNSAPISSNTLDTLLDKNQKTFNDFQ

SEQ ID NO: 8 - protein, 439 aa, Artificial Sequence
  Dda helicase
MTFDDLTEGQKNAFNIVMKAIKEKKHHVTINGPAGTGKTTLTKFIIEALISTGETGIILAAPTHAAKKILSKLSGKEASTIHSILKINPVTYEENVLFEQKEVPDLAKCRVLICDEVSMYDRKLFKILLSTIPPWCTIIGIGDNKQIRPVDPGENTAYISPFFTHKDFYQCELTEVKRSNAPIIDVATDVRNGKWIYDKVVDGHGVRGFTGDTALRDFMVNYFSIVKSLDDLFENRVMAFTNKSVDKLNSIIRKKIFETDKDFIVGEIIVMQEPLFKTYKIDGKPVSEIIFNNGQLVRIIEAEYTSTFVKARGVPGEYLIRHWDLTVETYGDDEYYREKIKIISSDEELYKFNLFLGKTAETYKNWNKGGKAPWSDFWDAKSQFSKVKALPASTFHKAQGMSVDRAFIYTPCIHYADVELAQQLLYVGVTRGRYDVFYV

SEQ ID NO: 9 - DNA, 16 bp, Artificial Sequence
  Tag oligo
ggaacctctctgacaa

SEQ ID NO: 10 - skipped

SEQ ID NO: 11 - DNA, 84 bp, Artificial Sequence
  Polynucleotide strand
  misc_feature (1)..(1): 5' phosphate
  misc_feature (30)..(31): 4iSp18
cgtcctgtcgctgtgtctcgttttttttttaatgtacttcgttcagttacgtattgctagagccgagacacagcgacaggacgt

SEQ ID NO: 12 - DNA, 45 bp, Artificial Sequence
  Polynucleotide strand
  misc_feature (1)..(1): 5' phosphate
  misc_feature (23)..(23): Bridged nucleic acid
  modified_base (24)..(24): m5c
  misc_feature (24)..(24): Bridged nucleic acid
  misc_feature (25)..(25): Bridged nucleic acid
  misc_feature (26)..(26): Bridged nucleic acid
  misc_feature (27)..(27): Bridged nucleic acid
gcaatacgtaactgaacgaagtacatttttgaggcgagcggtcaa

SEQ ID NO: 13 - DNA, 3595 bp, Artificial Sequence
  Polynucleotide analyte
gccatcagattgtgtttgttagtcgctgccatcagattgtgtttgttagtcgctttttttttttggaattttttttttggaattttttttttgcgctaacaacctcctgccgttttgcccgtgcatatcggtcacgaacaaatctgattactaaacacagtagcctggatttgttctatcagtaatcgaccttattcctaattaaatagagcaaatccccttattgggggtaagacatgaagatgccagaaaaacatgacctgttggccgccattctcgcggcaaaggaacaaggcatcggggcaatccttgcgtttgcaatggcgtaccttcgcggcagatataatggcggtgcgtttacaaaaacagtaatcgacgcaacgatgtgcgccattatcgcctagttcattcgtgaccttctcgacttcgccggactaagtagcaatctcgcttatataacgagcgtgtttatcggctacatcggtactgactcgattggttcgcttatcaaacgcttcgctgctaaaaaagccggagtagaagatggtagaaatcaataatcaacgtaaggcgttcctcgatatgctggcgtggtcggagggaactgataacggacgtcagaaaaccagaaatcatggttatgacgtcattgtaggcggagagctatttactgattactccgatcaccctcgcaaacttgtcacgctaaacccaaaactcaaatcaacaggcgccggacgctaccagcttctttcccgttggtgggatgcctaccgcaagcagcttggcctgaaagacttctctccgaaaagtcaggacgctgtggcattgcagcagattaaggagcgtggcgctttacctatgattgatcgtggtgatatccgtcaggcaatcgaccgttgcagcaatatctgggcttcactgccgggcgctggttatggtcagttcgagcataaggctgacagcctgattgcaaaattcaaagaagcgggcggaacggtcagagagattgatgtatgagcagagtcaccgcgattatctccgctctggttatctgcatcatcgtctgcctgtcatgggctgttaatcattaccgtgataacgccattacctacaaagcccagcgcgacaaaaatgccagagaactgaagctggcgaacgcggcaattactgacatgcagatgcgtcagcgtgatgttgctgcgctcgatgcaaaatacacgaaggagttagctgatgctaaagctgaaaatgatgctctgcgtgatgatgttgccgctggtcgtcgtcggttgcacatcaaagcagtctgtcagtcagtgcgtgaagccaccaccgcctccggcgtggataatgcagcctccccccgactggcagacaccgctgaacgggattatttcaccctcagagagaggctgatcactatgcaaaaacaactggaaggaacccagaagtatattaatgagcagtgcagatagagttgcccatatcgatgggcaactcatgcaattattgtgagcaatacacacgcgcttccagcggagtataaatgcctaaagtaataaaaccgagcaatccatttacgaatgtttgctgggtttctgttttaacaacattttctgcgccgccacaaattttggctgcatcgacagttttcttctgcccaattccagaaacgaagaaatgatgggtgatggtttcctttggtgctactgctgccggtttgttttgaacagtaaacgtctgttgagcacatcctgtaataagcagggccagcgcagtagcgagtagcatttttttcatggtgttattcccgatgctttttgaagttcgcagaatcgtatgtgtagaaaattaaacaaaccctaaacaatgagttgaaatttcatattgttaatatttattaatgtatgtcaggtgcgatgaatcgtcattgtattcccggattaactatgtccacagccctgacggggaacttctctgcgggagtgtccgggaataattaaaacgatgcacacagggtttagcgcgtacacgtattgcattatgccaacgccccggtgctgacacggaagaaaccggacgttatgatttagcgtggaaagatttgtgtagtgttctgaatgctctcagtaaatagtaatgaattatcaaaggtatagtaatatcttttatgttcatggatatttgtaacccatcggaaaactcctgctttagcaagattttccctgtattgctgaaatgtgatttctcttgatttcaacctatcataggacgtttctataagatgcgtgtttcttgagaatttaacatttacaacctttttaagtccttttattaacacggtgttatcgttttctaacacgatgtgaatattatctgtggctagatagtaaatataatgtgagacgttgtgacgttttagttcagaataaaacaattcacagtctaaatcttttcgcacttgatcgaatatttctttaaaaatggcaacctgagccattggtaaaaccttccatgtgatacgagggcgcgtagtttgcattatcgtttttatcgtttcaatctggtctgacctccttgtgttttgttgatgatttatgtcaaatattaggaatgttttcacttaatagtattggttgcgtaacaaagtgcggtcctgctggcattctggagggaaatacaaccgacagatgtatgtaaggccaacgtgctcaaatcttcatacagaaagatttgaagtaatattttaaccgctagatgaagagcaagcgcatggagcgacaaaatgaataaagaacaatctgctgatgatccctccgtggatctgattcgtgtaaaaaatatgcttaatagcaccatttctatgagttaccctgatgttgtaattgcatgtatagaacataaggtgtctctggaagcattcagagcaattgaggcagcgttggtgaagcacgataataatatgaaggattattccctggtggttgactgatcaccataactgctaatcattcaaactatttagtctgtgacagagccaacacgcagtctgtcactgtcaggaaagtggtaaaactgcaactcaattactgcaatgccctcgtaattaagtgaatttacaatatcgtcctgttcggagggaagaacgcgggatgttcattcttcatcacttttaattgatgtatatgctctcttttctgacgttagtctccgacggcaggcttcaatgacccaggctgagaaattcccggaccctttttgctcaagagcgatgttaatttgttcaatcatttggttaggaaagcggatgttgcgggttgttgttctgcgggttctgttcttcgttgacatgaggttgccccgtattcagtgtcgctgatttgtattgtctgaagttgtttttacgttaagttgatgcagatcaattaatacgatacctgcgtcataattgattatttgacgtggtttgatggcctccacgcacgttgtgatatgtagatgataatcattatcactttacgggtcctttccggtgaaaaaaaaggtaccaaaaaaaacatcgtcgtgagtagtgaaccgtaagcatgtagga

SEQ ID NO: 14 - DNA, 10126 bp, Artificial Sequence
  Polynucleotide analyte
ggtcaggttgtggtgattggtcgctgatgcaaaatgttttatgtgaaaccgcctgcgggcggttttgtcatttatggagcgtgaggaatgggtaaaggaagcagtaaggggcataccccgcgcgaagcgaaggacaacctaggagaagtccacgcagttgctgagtgtgatcgatgccatcagcgaagggccgattgaaggtccggtggatggcttaaaaagcgtgctgctgaacagtacgccggtgctggacactgaggggaataccaacatatccggtgtcacggtggtgttccgggctggtgagcaggagcagactccgccggagggatttgaatcctccggctccgagacggtgctgggtacggaagtgaaatatgacacgccgatcacccgcaccattacgtctgcaaacatcgaccgtctgcgctttaccttcggtgtacaggcactggtggaaaccacctcaaagggtgacaggaatccgtcggaagtccgcctgctggttcagatacaacgtaacggtggctgggtgacggaaaaagacatcaccattaagggcaaaaccacctcgcagtatctggcctcggtggtgatgggtaacctgccgccgcgcccgtttaatatccggatgcgcaggatgacgccggacagcaccacagaccagctgcagaacaaaacgctctggtcgtcatacactgaaatcatcgatgtgaaacagtgctacccgaacacggcactggtcggcgtgcaggtggactcggagcagttcggcagccagcaggtgagccgtaattatcatctgcgcgggcgtattctgcaggtgccgtcgaactataacccgcagacgcggcaatacagcggtatctgggacggaacgtttaaaccggcatacagcaacaacatggcctggtgtctgtgggatatgctgacccatccgcgctacggcatggggaaacgtcttggtgcggcggatgtggataaatgggcgctgtatgtcatcggccagtactgcgaccagtcagtgccggacggctttggcggcacggagccgcgcatcacctgtaatgcgtacctgaccacacagcgtaaggcgtgggatgtgctcagcgatttctgctcggcgatgcgctgtatgccggtatggaacgggcagacgctgacgttcgtgcaggaccgaccgtcggataagacgtggacctataaccgcagtaatgtggtgatgccggatgatggcgcgccgttccgctacagcttcagcgccctgaaggaccgccataatgccgttgaggtgaactggattgacccgaacaacggctgggagacggcgacagagcttgttgaagatacgcaggccattgcccgttacggtcgtaatgttacgaagatggatgcctttggctgtaccagccgggggcaggcacaccgcgccgggctgtggctgattaaaacagaactgctggaaacgcagaccgtggatttcagcgtcggcgcagaagggcttcgccatgtaccgggcgatgttattgaaatctgcgatgatgactatgccggtatcagcaccggtggtcgtgtgctggcggtgaacagccagacccggacgctgacgctcgaccgtgaaatcacgctgccatcctccggtaccgcgctgataagcctggttgacggaagtggcaatccggtcagcgtggaggttcagtccgtcaccgacggcgtgaaggtaaaagtgagccgtgttcctgacggtgttgctgaatacagcgtatgggagctgaagctgccgacgctgcgccagcgactgttccgctgcgtgagtatccgtgagaacgacgacggcacgtatgccatcaccgccgtgcagcatgtgccggaaaaagaggccatcgtggataacggggcgcactttgacggcgaacagagtggcacggtgaatggtgtcacgccgccagcggtgcagcacctgaccgcagaagtcactgcagacagcggggaatatcaggtgctggcgcgatgggacacaccgaaggtggtgaagggcgtgagtttcctgctccgtctgaccgtaacagcggacgacggcagtgagcggctggtcagcacggcccggacgacggaaaccacataccgcttcacgcaactggcgctggggaactacaggctgacagtccgggcggtaaatgcgtgggggcagcagggcgatccggcgtcggtatcgttccggattgccgcaccggcagcaccgtcgaggattgagctgacgccgggctattttcagataaccgccacgccgcatcttgccgtttatgacccgacggtacagtttgagttctggttctcggaaaagcagattgcggatatcagacaggttgaaaccagcacgcgttatcttggtacggcgctgtactggatagccgccagtatcaatatcaaaccgggccatgattattacttttatatccgcagtgtgaacaccgttggcaaatcggcattcgtggaggccgtcggtcgggcgagcgatgatgcggaaggttacctggattttttcaaaggcaagataaccgaatcccatctcggcaaggagctgctggaaaaagtcgagctgacggaggataacgccagcagactggaggagttttcgaaagagtggaaggatgccagtgataagtggaatgccatgtgggctgtcaaaattgagcagaccaaagacggcaaacattatgtcgcgggtattggcctcagcatggaggacacggaggaaggcaaactgagccagtttctggttgccgccaatcgtatcgcatttattgacccggcaaacgggaatgaaacgccgatgtttgtggcgcagggcaaccagatattcatgaacgacgtgttcctgaagcgcctgacggcccccaccattaccagcggcggcaatcctccggccttttccctgacaccggacggaaagctgaccgctaaaaatgcggatatcagtggcagtgtgaatgcgaactccgggacgctcagtaatgtgacgatagctgaaaactgtacgataaacggtacgctgagggcggaaaaaatcgtcggggacattgtaaaggcggcgagcgcggcttttccgcgccagcgtgaaagcagtgtggactggccgtcaggtacccgtactgtcaccgtgaccgatgaccatccttttgatcgccagatagtggtgcttccgctgacgtttcgcggaagtaagcgtactgtcagcggcaggacaacgtattcgatgtgttatctgaaagtactgatgaacggtgcggtgatttatgatggcgcggcgaacgaggcggtacaggtgttctcccgtattgttgacatgccagcgggtcggggaaacgtgatcctgacgttcacgcttacgtccacacggcattcggcagatattccgccgtatacgtttgccagcgatgtgcaggttatggtgattaagaaacaggcgctgggcatcagcgtggtctgagtgtgttacagaggttcgtccgggaacgggcgttttattataaaacagtgagaggtgaacgatgcgtaatgtgtgtattgccgttgctgtctttgccgcacttgcggtgacagtcactccggcccgtgcggaaggtggacatggtacgtttacggtgggctattttcaagtgaaaccgggtacattgccgtcgttgtcgggcggggataccggtgtgagtcatctgaaagggattaacgtgaagtaccgttatgagctgacggacagtgtgggggtgatggcttccctggggttcgccgcgtcgaaaaagagcagcacagtgatgaccggggaggatacgtttcactatgagagcctgcgtggacgttatgtgagcgtgatggccggaccggttttacaaatcagtaagcaggtcagtgcgtacgccatggccggagtggctcacagtcggtggtccggcagtacaatggattaccgtaagacggaaatcactcccgggtatatgaaagagacgaccactgccagggacgaaagtgcaatgcggcatacctcagtggcgtggagtgcaggtatacagattaatccggcagcgtccgtcgttgttgatattgcttatgaaggctccggcagtggcgactggcgtactgacggattcatcgttggggtcggttataaattctgattagccaggtaacacagtgttatgacagcccgccggaaccggtgggcttttttgtggggtgaatatggcagtaaagatttcaggagtcctgaaagacggcacaggaaaaccggtacagaactgcaccattcagctgaaagccagacgtaacagcaccacggtggtggtgaacacggtgggctcagagaatccggatgaagccgggcgttacagcatggatgtggagtacggtcagtacagtgtcatcctgcaggttgacggttttccaccatcgcacgccgggaccatcaccgtgtatgaagattcacaaccggggacgctgaatgattttctctgtgccatgacggaggatgatgcccggccggaggtgctgcgtcgtcttgaactgatggtggaagaggtggcgcgtaacgcgtccgtggtggcacagagtacggcagacgcgaagaaatcagccggcgatgccagtgcatcagctgctcaggtcgcggcccttgtgactgatgcaactgactcagcacgcgccgccagcacgtccgccggacaggctgcatcgtcagctcaggaagcgtcctccggcgcagaagcggcatcagcaaaggccactgaagcggaaaaaagtgccgcagccgcagagtcctcaaaaaacgcggcggccaccagtgccggtgcggcgaaaacgtcagaaacgaatgctgcagcgtcacaacaatcagccgccacgtctgcctccaccgcggccacgaaagcgtcagaggccgccacttcagcacgagatgcggtggcctcaaaagaggcagcaaaatcatcagaaacgaacgcatcatcaagtgccggtcgtgcagcttcctcggcaacggcggcagaaaattctgccagggcggcaaaaacgtccgagacgaatgccaggtcatctgaaacagcagcggaacggagcgcctctgccgcggcagacgcaaaaacagcggcggcggggagtgcgtcaacggcatccacgaaggcgacagaggctgcgggaagtgcggtatcagcatcgcagagcaaaagtgcggcagaagcggcggcaatacgtgcaaaaaattcggcaaaacgtgcagaagatatagcttcagctgtcgcgcttgaggatgcggacacaacgagaaaggggatagtgcagctcagcagtgcaaccaacagcacgtctgaaacgcttgctgcaacgccaaaggcggttaaggtggtaatggatgaaacgaacagaaaagcccactggacagtccggcactgaccggaacgccaacagcaccaaccgcgctcaggggaacaaacaatacccagattgcgaacaccgcttttgtactggccgcgattgcagatgttatcgacgcgtcacctgacgcactgaatacgctgaatgaactggccgcagcgctcgggaatgatccagattttgctaccaccatgactaacgcgcttgcgggtaaacaaccgaagaatgcgacactgacggcgctggcagggctttccacggcgaaaaataaattaccgtattttgcggaaaatgatgccgccagcctgactgaactgactcaggttggcagggatattctggcaaaaaattccgttgcagatgttcttgaataccttggggccggtgagaattcggcctttccggcaggtgcgccgatcccgtggccatcagatatcgttccgtctggctacgtcctgatgcaggggcaggcgtttgacaaatcagcctacccaaaacttgctgtcgcgtatccatcgggtgtgcttcctgatatgcgaggctggacaatcaaggggaaacccgccagcggtcgtgctgtattgtctcaggaacaggatggaattaagtcgcacacccacagtgccagtgcatccggtacggatttggggacgaaaaccacatcgtcgtttgattacgggacgaaaacaacaggcagtttcgattacggcaccaaatcgacgaataacacgggggctcatgctcacagtctgagcggttcaacaggggccgcgggtgctcatgcccacacaagtggtttaaggatgaacagttctggctggagtcagtatggaacagcaaccattacaggaagtttatccacagttaaaggaaccagcacacagggtattgcttatttatcgaaaacggacagtcagggcagccacagtcactcattgtccggtacagccgtgagtgccggtgcacatgcgcatacagttggtattggtgcgcaccagcatccggttgttatcggtgctcatgcccattctttcagtattggttcacacggacacaccatcaccgttaacgctgcgggtaacgcggaaaacaccgtcaaaaacattgcatttaactatattgtgaggcttgcataatggcattcagaatgagtgaacaaccacggaccataaaaatttataatctgctggccggaactaatgaatttattggtgaaggtgacgcatatattccgcctcataccggtctgcctgcaaacagtaccgatattgcaccgccagatattccggctggctttgtggctgttttcaacagtgatgaggcatcgtggcatctcgttgaagaccatcggggtaaaaccgtctatgacgtggcttccggcgacgcgttatttatttctgaactcggtccgttaccggaaaattttacctggttatcgccgggaggggaatatcagaagtggaacggcacagcctgggtgaaggatacggaagcagaaaaactgttccggatccgggaggcggaagaaacaaaaaaaagcctgatgcaggtagccagtgagcatattgcgccgcttcaggatgctgcagatctggaaattgcaacgaaggaagaaacctcgttgctggaagcctggaagaagtatcgggtgttgctgaaccgtgttgatacatcaactgcacctgatattgagtggcctgctgtccctgttatggagtaatcgttttgtgatatgccgcagaaacgttgtatgaaataacgttctgcggttagttagtatattgtaaagctgagtattggtttatttggcgattattatcttcaggagaataatggaagttctatgactcaattgttcatagtgtttacatcaccgccaattgcttttaagactgaacgcatgaaatatggtttttcgtcatgttttgagtctgctgttgatatttctaaagtcggttttttttcttcgttttctctaactattttccatgaaatacatttttgattattatttgaatcaattccaattacctgaagtctttcatctataattggcattgtatgtattggtttattggagtagatgcttgcttttctgagccatagctctgatatccaaatgaagccataggcatttgttattttggctctgtcagctgcataacgccaaaaaatatatttatctgcttgatcttcaaatgttgtattgattaaatcaattggatggaattgtttatcataaaaaattaatgtttgaatgtgataaccgtcctttaaaaaagtcgtttctgcaagcttggctgtatagtcaactaactcttctgtcgaagtgatatttttaggcttatctaccagttttagacgctctttaatatcttcaggaattattttattgtcatattgtatcatgctaaatgacaatttgcttatggagtaatcttttaattttaaataagttattctcctggcttcatcaaataaagagtcgaatgatgttggcgaaatcacatcgtcacccattggattgtttatttgtatgccaagagagttacagcagttatacattctgccatagattatagctaaggcatgtaataattcgtaatcttttagcgtattagcgacccatcgtctttctgatttaataatagatgattcagttaaatatgaaggtaatttcttttgtgcaagtctgactaacttttttataccaatgtttaacatactttcatttgtaataaactcaatgtcattttcttcaatgtaagatgaaataagagtagcctttgcctcgctatacatttctaaatcgccttgtttttctatcgtattgcgagaatttttagcccaagccattaatggatcatttttccatttttcaataacattattgttataccaaatgtcatatcctataatctggtttttgtttttttgaataataaatgttactgttcttgcggtttggaggaattgattcaaattcaagcgaaataattcagggtcaaaatatgtatcaatgcagcatttgagcaagtgcgataaatctttaagtcttctttcccatggttttttagtcataaaactctccattttgataggttgcatgctagatgctgatatattttagaggtgataaaattaactgcttaactgtcaatgtaatacaagttgtttgatctttgcaatgattcttatcagaaaccatatagtaaattagttacacaggaaatttttaatattattattatcattcattatgtattaaaattagagttgtggcttggctctgctaacacgttgctcataggagatatggtagagccgcagacacgtcgtatgcaggaacgtgctgcggctggctggtgaacttccgatagtgcgggtgttgaatgatttccagttgctaccgattttacatattttttgcatgagagaatttgtaccacctcccaccgaccatctatgactgtacgccactgtccctaggactgctatgtgccggagcggacattacaaacgtccttctcggtgcatgccactgttgccaatgacctgcctaggaattggttagcaagttactaccggattttgtaaaaacagccctcctcatataaaaagtattcgttcacttccgataagcgtcgtaattttctatctttcatcatattctagatccctctgaaaaaatcttccgagtttgctaggcactgatacataactcttttccaataattggggaagtcattcaaatctataataggtttcagatttgcttcaataaattctgactgtagctgctgaaacgttgcggttgaactatatttccttataacttttacgaaagagtttctttgagtaatcacttcactcaagtgcttccctgcctccaaacgatacctgttagcaatatttaatagcttgaaatgatgaagagctctgtgtttgtcttcctgcctccagttcgccgggcattcaacataaaaactgatagcacccggagttccggaaacgaaatttgcatatacccattgctcacgaaaaaaaatgtccttgtcgatatagggatgaatcgcttggtgtacctcatctactgcgaaaacttgacctttctctcccatattgcagtcgcggcacgatggaactaaattaataggcatcaccgaaaattcaggataatgtgcaataggaagaaaatgatctatattttttgtctgtcctatatcaccacaaaatggacatttttcacctgatgaaacaagcatgtcatcgtaatatgttctagcgggtttgtttttatctcggagattattttcataaagcttttctaatttaacctttgtcaggttaccaactactaaggttgtaggctcaagagggtgtgtcctgtcgtaggtaaataactgacctgtcgagcttaatattctatattgttgttctttctgcaaaaaagtggggaagtgagtaatgaaattatttctaacatttatctgcatcataccttccgagcatttattaagcatttcgctataagttctcgctggaagaggtagttttttcattgtactttaccttcatctctgttcattatcatcgcttttaaaacggttcgaccttctaatcctatctgaccattataattttttagaatggtttcataagaaagctctgaatcaacggactgcgataataagtggtagga

SEQ ID NO: 15 - DNA, 41 bp, Artificial Sequence
  Polynucleotide adapter
ggttaaacacccaagcagacgcctttgaggcgagcggtcaa

SEQ ID NO: 16 - DNA, 44 bp, Artificial Sequence
  Polynucleotide adapter
  misc_feature (1)..(1): 20iSpC3
  misc_feature (10)..(11): 10iSpC3
ttttttttttttttttttttggcgtctgcttgggtgtttaacct

SEQ ID NO: 17-19 - skipped (3 entries)

SEQ ID NO: 20 - DNA, 3595 bp, Artificial Sequence; identical to SEQ ID NO: 13
  Bacteriophage lambda fragment

SEQ ID NO: 21 - DNA, 38 bp, Artificial Sequence
  Oligo
  misc_feature (1)..(1): 5' biotin, via TEG linker
  misc_feature (10)..(11): iSp18
ttttttttttaatgtacttcgttcagttacgtattgct

SEQ ID NO: 22 - DNA, 65 bp, Artificial Sequence
  Oligo
  misc_feature (1)..(1): 5' phosphate
  misc_feature (23)..(23): Bridged nucleic acid
  modified_base (24)..(24): m5c
  misc_feature (24)..(24): Bridged nucleic acid
  misc_feature (25)..(25): Bridged nucleic acid
  misc_feature (26)..(26): Bridged nucleic acid
  misc_feature (27)..(27): Bridged nucleic acid
gcaatacgtaactgaacgaagtacatttttgaggcgagcggtcaatttttttttttttttttttt

SEQ ID NO: 23 - skipped

SEQ ID NO: 24 - DNA, 91 bp, Artificial Sequence
  Hairpin oligo
  misc_feature (1)..(1): 5' phosphate
tgcaatacgtaactgaacgaagtacatttttttgaagatagagcgattttttttttttttttgtacttcgttcagttacgtattgcatcct

SEQ ID NO: 25 - DNA, 88 bp, Artificial Sequence
  Hairpin oligo
  misc_feature (1)..(1): 5' phosphate
tgcaatacgtaactgaacgaagtacatttttttgaagatagagcgattttttttttttttttgtacttcgttcagttacgtattgcat

SEQ ID NO: 26 - DNA, 92 bp, Artificial Sequence
  Hairpin oligo
  misc_feature (1)..(1): 5' phosphate
  misc_feature (52)..(52): 5' fluorescein
  misc_feature (53)..(53): 5' fluorescein
  misc_feature (54)..(54): 5' fluorescein
tgcaatacgtaactgaacgaagtacatttttttgaagatagagcgatttttttttttttttttgtacttcgttcagttacgtattgcatcct

SEQ ID NO: 27 - DNA, 13 bp, Artificial Sequence
  Oligo
  misc_feature (1)..(1): Bridged nucleic acid
  modified_base (2)..(2): m5c
  misc_feature (2)..(2): Bridged nucleic acid
  misc_feature (3)..(3): Bridged nucleic acid
  modified_base (4)..(4): m5c
  misc_feature (4)..(4): Bridged nucleic acid
  misc_feature (5)..(5): Bridged nucleic acid
tcgctctatcttc

SEQ ID NO: 28 - DNA, 89 bp, Artificial Sequence
  Y-adapter oligo
  misc_feature (35)..(36): iSp18
gttattcaagacttctttaatacacttttttttttaatgtacttcgttcagttacgtattgctttggcgtctgcttgggtgtttaacct

SEQ ID NO: 29 - skipped

SEQ ID NO: 30 - DNA, 27 bp, Artificial Sequence
  Y-adapter oligo
  misc_feature (23)..(23): Bridged nucleic acid
  modified_base (24)..(24): m5c
  misc_feature (24)..(24): Bridged nucleic acid
  misc_feature (25)..(25): Bridged nucleic acid
  misc_feature (26)..(26): Bridged nucleic acid
  misc_feature (27)..(27): Bridged nucleic acid
gcaatacgtaactgaacgaagtacatt

SEQ ID NO: 31 - skipped

SEQ ID NO: 32 - DNA, 25 bp, Artificial Sequence
  Y-adapter oligo
gtgtattaaagaagtcttgaataac

SEQ ID NO: 33 - DNA, 41 bp, Artificial Sequence; identical to SEQ ID NO: 15
  Y-adapter oligo
  misc_feature (1)..(1): 5' phosphate
  misc_feature (41)..(41): 30iSpC3

SEQ ID NO: 34 - DNA, 89 bp, Artificial Sequence; identical to SEQ ID NO: 28
  Y-adapter oligo
  misc_feature (36)..(37): iSp9

SEQ ID NO: 35 - DNA, 21 bp, Artificial Sequence
  Y-adapter oligo
  misc_feature (1)..(1): 5' phosphate
  misc_feature (21)..(21): 30iSpC3
aacacccaagcagacgccttt

SEQ ID NO: 36 - DNA, 30 bp, Artificial Sequence
  Y-adapter oligo
  misc_feature (26)..(26): Bridged nucleic acid
  modified_base (27)..(27): m5c
  misc_feature (27)..(27): Bridged nucleic acid
  misc_feature (28)..(28): Bridged nucleic acid
  misc_feature (29)..(29): Bridged nucleic acid
  misc_feature (30)..(30): Bridged nucleic acid
tttgcaatacgtaactgaacgaagtacatt

SEQ ID NO: 37 - DNA, 37 bp, Artificial Sequence
  Y-adapter oligo
  misc_feature (26)..(27): 3iSpC3
  misc_feature (37)..(37): 3' dideoxycytidine
gtgtattaaagaagtcttgaataacgaggcgagcggt

SEQ ID NO: 38 - DNA, 50 bp, Artificial Sequence
  Transposase adapter oligo
  misc_feature (1)..(1): 5' phosphate
gttttcgcatttatcgtgaaacgctttcgcgtttttcgtgcgccgcttca

SEQ ID NO: 39 - DNA, 61 bp, Artificial Sequence
  Transposase adapter oligo
  misc_feature (1)..(1): 5' phosphate
  misc_feature (1)..(5): n is inosine
nnnnntgaagcggcgcacgaaaaacgcgaaagcgtttcacgataaatgcgaaaacaggtta

SEQ ID NO: 40 - DNA, 84 bp, Artificial Sequence; identical to SEQ ID NO: 11
  Hairpin adapter oligo
  misc_feature (1)..(1): 5' phosphate
  misc_feature (20)..(21): 10iSpC3
  misc_feature (30)..(31): iSp18

SEQ ID NO: 41 - DNA, 27 bp, Artificial Sequence
  Hairpin adapter oligo
  misc_feature (23)..(23): Bridged nucleic acid
  modified_base (24)..(24): m5c
  misc_feature (24)..(24): Bridged nucleic acid
  misc_feature (25)..(25): Bridged nucleic acid
  misc_feature (26)..(26): Bridged nucleic acid
  misc_feature (27)..(27): Bridged nucleic acid
gcaatacgtaactgaacgaagtacatt

SEQ ID NO: 42 - DNA, 61 bp, Artificial Sequence
  Leader adapter oligo
  misc_feature (1)..(1): 30iSpC3
  misc_feature (33)..(34): iSp18
  misc_feature (61)..(61): 3' amino C7 labelled with azidohexanoic acid
ctacatctccttattcgctgcacttttttttttcctgtacttcgttcagttacgtattgct

SEQ ID NO: 43 - DNA, 41 bp, Artificial Sequence
  Leader adapter oligo
gtgcagcgaataaggagatgtagtttgaggcgagcggtcaa

SEQ ID NO: 44 - DNA, 45 bp, Artificial Sequence
  Leader adapter oligo
  modified_base (36)..(36): gm
  misc_feature (37)..(37): 2-O-methyladenosine
  misc_feature (38)..(38): 2-O-methyladenosine
  modified_base (39)..(39): gm
  modified_base (40)..(40): um
  misc_feature (41)..(41): 2-O-methyladenosine
  modified_base (42)..(42): cm
  misc_feature (43)..(43): 2-O-methyladenosine
  modified_base (44)..(44): gm
  modified_base (45)..(45): gm
ggttaaacacccaagcaagcaatacgtaactgaacgaaguacagg

SEQ ID NO: 45 - DNA, 30 bp, Artificial Sequence
  Leader adapter oligo
gcaatacgtaactgaacgaagtacaggttt

SEQ ID NO: 46 - DNA, 26 bp, Artificial Sequence
  Leader adapter oligo
  misc_feature (1)..(1): 5' phosphate
  misc_feature (26)..(26): 30iSpC3
ggttaaacacccaagcagacgccttt

SEQ ID NO: 47 - DNA, 50 bp, Artificial Sequence; identical to SEQ ID NO: 38
  Transposase adapter oligo
  misc_feature (1)..(1): 5' phosphate